European Patent Specification EP 4 032 978 B1, published January 29, 2025. Title: CD19-Targeted Chimeric Antigen Receptor and Use Thereof. Applicant: JUVENTAS CELL THERAPY LTD. The sequence listing filed with the application follows.

SEQUENCE LISTING (2 sequences)

SEQ ID NO: 1 - protein, 493 aa, Artificial Sequence
  Tn Amino Acid Sequence of The Chimeric Antigen Receptor
MALPVTALLLPLALLLHAARPGSDIVLTQSPKFMSTSVGDRVSVTCKASQNVGTNVAWYQQKPGQSPKPLIYSATYRNSGVPDRFTGSGSGTDFTLTITNVQSKDLADYFCQQYNRYPYTSGGGTKLEIKRGGGGSGGGGSGGGGSQVQLQQSGAELVRPGSSVKISCKASGYAFSSYWMNWVKQRPGQGLEWIGQIYPGDGDTNYNGKFKGQATLTADKSSSTAYMQLSGLTSEDSAVYFCARKTISSVVDFYFDYWGQGTTLTVSSEFTTTPAPRPPTPAPTIASQPLSLRPEACRPAAGGAVHTRGLDFACDIYIWAPLAGTCGVLLLSLVITLYCKRGRKKLLYIFKQPFMRPVQTTQEEDGCSCRFPEEEEGGCELRVKFSRSADAPAYQQGQNQLYNELNLGRREEYDVLDKRRGRDPEMGGKPRRKNPQEGLYNELQKDKMAEAYSEIGMKGERRRGKGHDGLYQGLSTATKDTYDALHMQALPPR

SEQ ID NO: 2 - DNA, 1482 bp, Artificial Sequence
  The Nucleic Acid Sequence Ecoding The Chimeric Antigen Receptor
atggccttaccagtgaccgccttgctcctgccgctggccttgctgctccacgccgccaggccgggatccgatattgtgctgacccagagccccaagttcatgagcaccagcgtgggcgatagagtgagcgtgacctgcaaggcaagccagaacgtgggaacaaacgtggcctggtaccaacagaaacccggccaaagccctaagcccctgatttacagcgccacctacagaaatagcggcgtgcccgacagatttacaggaagcggcagcggaaccgatttcacactgaccatcaccaacgtgcagagcaaagacctggccgactacttctgccagcagtacaacagatacccctacaccagcggaggaggaacaaagctggagatcaagagaggtggtggtggttctggcggcggcggctccggtggtggtggttctcaagtgcaactgcaacagagcggagccgaactggtgagacccggaagcagcgtgaagatcagctgcaaggcttccggctacgcctttagcagctactggatgaactgggtgaagcagagacctggacagggactggaatggatcggccagatttaccctggagacggcgacacaaactacaacggcaagttcaagggccaagctacactgaccgccgacaaaagcagcagcaccgcctatatgcagctgagcggactgaccagcgaagatagcgctgtgtacttctgcgccagaaagaccatcagcagcgtggtggacttctacttcgactactggggacaaggcaccaccctgacagtgagcagcgaattcaccacgacgccagcgccgcgaccaccaacaccggcgcccaccatcgcgtcgcagcccctgtccctgcgcccagaggcgtgccggccagcggcggggggcgcagtgcacacgagggggctggacttcgcctgtgatatctacatctgggcgcccttggccgggacttgtggggtccttctcctgtcactggttatcaccctttactgcaaacggggcagaaagaaactcctgtatatattcaaacaaccatttatgagaccagtacaaactactcaagaggaagatggctgtagctgccgatttccagaagaagaagaaggaggatgtgaactgagagtgaagttcagcaggagcgcagacgcccccgcgtaccagcagggccagaaccagctctataacgagctcaatctaggacgaagagaggagtacgatgttttggacaagagacgtggccgggaccctgagatggggggaaagccgagaaggaagaaccctcaggaaggcctgtacaatgaactgcagaaagataagatggcggaggcctacagtgagattgggatgaaaggcgagcgccggaggggcaaggggcacgatggcctttaccagggtctcagtacagccaccaaggacacctacgacgcccttcacatgcaggccctgccccctcgctaa